European Patent Application EP 4 621 072 A1, published September 24, 2025. Title: METHOD FOR DETECTING METHYLATION STATUS OF DNA SAMPLE. Applicant: NANODIGMBIO (NANJING) BIOTECHNOLOGY CO., LTD. The sequence listing filed with the application follows.

SEQUENCE LISTING (219 sequences)

SEQ ID NO: 1 - DNA, 52 bp, synthetic construct
  source 1..52: mol_type = other DNA; note = Probe sequence
cgtcggtcgggagagcggtgggaagtattcgcctccgttcctcacaccgacg

SEQ ID NO: 2 - DNA, 50 bp, synthetic construct
  source 1..50: mol_type = other DNA; note = Probe sequence
cgtcggtcgacaggatgcgagcgccctttggagaagtcgcgccaccgacg

SEQ ID NO: 3 - DNA, 51 bp, synthetic construct
  source 1..51: mol_type = other DNA; note = Probe sequence
cgtcggtcggcggaaacgctaactccccggccaagtgcaaatgcaccgacg

SEQ ID NO: 4 - DNA, 52 bp, synthetic construct
  source 1..52: mol_type = other DNA; note = Probe sequence
cgtcggtcggcacacacgagggcccgtcgcgccccccgccctgccaccgacg

SEQ ID NO: 5 - DNA, 51 bp, synthetic construct
  source 1..51: mol_type = other DNA; note = Probe sequence
cgtcggtcggcctcgccctccacgtccctgcacccccaagtcgcaccgacg

SEQ ID NO: 6 - DNA, 51 bp, synthetic construct
  source 1..51: mol_type = other DNA; note = Probe sequence
cgtcggtcgtaagaacccagtccccgatcggtttcctctacgccaccgacg

SEQ ID NO: 7 - DNA, 51 bp, synthetic construct
  source 1..51: mol_type = other DNA; note = Probe sequence
cgtcggtcgggagggagggggggaaagggggacgaggggcggacaccgacg

SEQ ID NO: 8 - DNA, 52 bp, synthetic construct
  source 1..52: mol_type = other DNA; note = Probe sequence
cgtcggtcgggggggtttggaagcgcactgccacttgcaaagtccaccgacg

SEQ ID NO: 9 - DNA, 52 bp, synthetic construct
  source 1..52: mol_type = other DNA; note = Probe sequence
cgtcggtcgacccgagcaatcacagccggagcgcgattcgaatgcaccgacg

SEQ ID NO: 10 - DNA, 51 bp, synthetic construct
  source 1..51: mol_type = other DNA; note = Probe sequence
cgtcggtcgtgaaccgaagacctcgtaggcgggcctcggggggcaccgacg

SEQ ID NO: 11 - DNA, 52 bp, synthetic construct
  source 1..52: mol_type = other DNA; note = Probe sequence
cgtcggtcggatgccgttggcggcggccagcgccagcccctcggcaccgacg

SEQ ID NO: 12 - DNA, 51 bp, synthetic construct
  source 1..51: mol_type = other DNA; note = Probe sequence
cgtcggtcggtgccgtagagcagctgcagctcgcgcgcctcgtcaccgacg

SEQ ID NO: 13 - DNA, 51 bp, synthetic construct
  source 1..51: mol_type = other DNA; note = Probe sequence
cgtcggtcgggctcaggtcgccgcagcccgggagcctccccgccaccgacg

SEQ ID NO: 14 - DNA, 51 bp, synthetic construct
  source 1..51: mol_type = other DNA; note = Probe sequence
cgtcggtcggccccaaggcacgcgcggcacagccatgaacacccaccgacg

SEQ ID NO: 15 - DNA, 51 bp, synthetic construct
  source 1..51: mol_type = other DNA; note = Probe sequence
cgtcggtcggatgccaaggagtatctggcccggagggaaatcccaccgacg

SEQ ID NO: 16 - DNA, 51 bp, synthetic construct
  source 1..51: mol_type = other DNA; note = Probe sequence
cgtcggtcggagtcccgcgcgctctccgtgcgccccggccggccaccgacg

SEQ ID NO: 17 - DNA, 52 bp, synthetic construct
  source 1..52: mol_type = other DNA; note = Probe sequence
cgtcggtcggcggcggctgccgcgcacaggcttccgactccagccaccgacg

SEQ ID NO: 18 - DNA, 51 bp, synthetic construct
  source 1..51: mol_type = other DNA; note = Probe sequence
cgtcggtcgcggcccgccactgagcatgcccagcacgccggcccaccgacg

SEQ ID NO: 19 - DNA, 52 bp, synthetic construct
  source 1..52: mol_type = other DNA; note = Probe sequence
cgtcggtcggagcggaggggacagcggggatcgtgagctccggccaccgacg

SEQ ID NO: 20 - DNA, 52 bp, synthetic construct
  source 1..52: mol_type = other DNA; note = Probe sequence
cgtcggtcggggcgagcgggtgcgtctgccgcagagtcggcacccaccgacg

SEQ ID NO: 21 - DNA, 52 bp, synthetic construct
  source 1..52: mol_type = other DNA; note = Probe sequence
cgtcggtcgaaggacatggaggtaaaggaccccggagggagacgcaccgacg

SEQ ID NO: 22 - DNA, 52 bp, synthetic construct
  source 1..52: mol_type = other DNA; note = Probe sequence
cgtcggtcggcacgtgcggcgctcagcttaggctctcggaggcacaccgacg

SEQ ID NO: 23 - DNA, 52 bp, synthetic construct
  source 1..52: mol_type = other DNA; note = Probe sequence
cgtcggtcgtgagttggaaatcccgacggaaagcacccacaagccaccgacg

SEQ ID NO: 24 - DNA, 51 bp, synthetic construct
  source 1..51: mol_type = other DNA; note = Probe sequence
cgtcggtcgcactctgcgctggcccacccgcgtgcacgcccaccaccgacg

SEQ ID NO: 25 - DNA, 51 bp, synthetic construct
  source 1..51: mol_type = other DNA; note = Probe sequence
cgtcggtcggcggagctaagcaggggtgtttggaaggcgcccgcaccgacg

SEQ ID NO: 26 - DNA, 50 bp, synthetic construct
  source 1..50: mol_type = other DNA; note = Probe sequence
cgtcggtcggctgtttgactgcgtggcttcacttggcccgcgcaccgacg

SEQ ID NO: 27 - DNA, 52 bp, synthetic construct
  source 1..52: mol_type = other DNA; note = Probe sequence
cgtcggtcgatcagcctctctggcgggggattctccccggactccaccgacg

SEQ ID NO: 28 - DNA, 52 bp, synthetic construct
  source 1..52: mol_type = other DNA; note = Probe sequence
cgtcggtcgggcgggcggggagccaggcccgagctgcgttctgccaccgacg

SEQ ID NO: 29 - DNA, 51 bp, synthetic construct
  source 1..51: mol_type = other DNA; note = Probe sequence
cgtcggtcgagccattggtgggcgccgcgctctgcactgagcacaccgacg

SEQ ID NO: 30 - DNA, 52 bp, synthetic construct
  source 1..52: mol_type = other DNA; note = Probe sequence
cgtcggtcgtcgcgccccgccggcccctagccgcagccgcagcccaccgacg

SEQ ID NO: 31 - DNA, 52 bp, synthetic construct
  source 1..52: mol_type = other DNA; note = Probe sequence
cgtcggtcgggcaggcggcaggacggggatcccaggctgcggggcaccgacg

SEQ ID NO: 32 - DNA, 52 bp, synthetic construct
  source 1..52: mol_type = other DNA; note = Probe sequence
cgtcggtcgactccgcggcagagccgctgggacctgacccgggacaccgacg

SEQ ID NO: 33 - DNA, 52 bp, synthetic construct
  source 1..52: mol_type = other DNA; note = Probe sequence
cgtcggtcggccttcgtccccgcgcgcacctccccgggtcgggccaccgacg

SEQ ID NO: 34 - DNA, 50 bp, synthetic construct
  source 1..50: mol_type = other DNA; note = Probe sequence
cgtcggtcgaaggggggctggtggaatctggcggtccccagccaccgacg

SEQ ID NO: 35 - DNA, 51 bp, synthetic construct
  source 1..51: mol_type = other DNA; note = Probe sequence
cgtcggtcgcgtgtcccgggtcggtgcgctcggcgcacccgtgcaccgacg

SEQ ID NO: 36 - DNA, 52 bp, synthetic construct
  source 1..52: mol_type = other DNA; note = Probe sequence
cgtcggtcggacagtgcccggcgtctgctcccacccgcccgccccaccgacg

SEQ ID NO: 37 - DNA, 52 bp, synthetic construct
  source 1..52: mol_type = other DNA; note = Probe sequence
cgtcggtcggaacttgccggtggtggggtcgtagtggtttccgacaccgacg

SEQ ID NO: 38 - DNA, 52 bp, synthetic construct
  source 1..52: mol_type = other DNA; note = Probe sequence
cgtcggtcgttggtgaccacgtcgtcgaacttgagcacctcgtacaccgacg

SEQ ID NO: 39 - DNA, 51 bp, synthetic construct
  source 1..51: mol_type = other DNA; note = Probe sequence
cgtcggtcgttcatgctgccgcttgaggccggcgtagaaggcgcaccgacg

SEQ ID NO: 40 - DNA, 51 bp, synthetic construct
  source 1..51: mol_type = other DNA; note = Probe sequence
cgtcggtcgggcggcccgggcaccgcgagccggccgagctccacaccgacg

SEQ ID NO: 41 - DNA, 51 bp, synthetic construct
  source 1..51: mol_type = other DNA; note = Probe sequence
cgtcggtcgggagctacgtgactacgtccacccgcacctacagcaccgacg

SEQ ID NO: 42 - DNA, 52 bp, synthetic construct
  source 1..52: mol_type = other DNA; note = Probe sequence
cgtcggtcgtgggcagcgcgctgcgccccagcaccagccgcagccaccgacg

SEQ ID NO: 43 - DNA, 52 bp, synthetic construct
  source 1..52: mol_type = other DNA; note = Probe sequence
cgtcggtcgggcgccgggcccgcgatcggagccggaggcaccgccaccgacg

SEQ ID NO: 44 - DNA, 52 bp, synthetic construct
  source 1..52: mol_type = other DNA; note = Probe sequence
cgtcggtcgagcggaaagagggctccgcggcggccaggctcagccaccgacg

SEQ ID NO: 45 - DNA, 52 bp, synthetic construct
  source 1..52: mol_type = other DNA; note = Probe sequence
cgtcggtcgtgccgggaaaatgctggatttaactcccagtctgccaccgacg

SEQ ID NO: 46 - DNA, 51 bp, synthetic construct
  source 1..51: mol_type = other DNA; note = Probe sequence
cgtcggtcgtcccggggatgccagactcctggggacgctgggacaccgacg

SEQ ID NO: 47 - DNA, 50 bp, synthetic construct
  source 1..50: mol_type = other DNA; note = Probe sequence
cgtcggtcggcggcgcggcgggacacgcaggactcccgcctccaccgacg

SEQ ID NO: 48 - DNA, 52 bp, synthetic construct
  source 1..52: mol_type = other DNA; note = Probe sequence
cgtcggtcggcccggaattcgttgagacggaatctcagcggatccaccgacg

SEQ ID NO: 49 - DNA, 52 bp, synthetic construct; identical to SEQ ID NO: 48
  source 1..52: mol_type = other DNA; note = Probe sequence

SEQ ID NO: 50 - DNA, 52 bp, synthetic construct
  source 1..52: mol_type = other DNA; note = Probe sequence
cgtcggtcgagatggccctgtcccggcgccccaggtcgtcgcgccaccgacg

SEQ ID NO: 51 - DNA, 52 bp, synthetic construct
  source 1..52: mol_type = other DNA; note = Probe sequence
cgtcggtcggcagctgcggtagtcactgcgcctccccgcccccacaccgacg

SEQ ID NO: 52 - DNA, 51 bp, synthetic construct
  source 1..51: mol_type = other DNA; note = Probe sequence
cgtcggtcgctggatgccccccttccctctcccggccagactccaccgacg

SEQ ID NO: 53 - DNA, 50 bp, synthetic construct
  source 1..50: mol_type = other DNA; note = Probe sequence
cgtcggtcgcggtgctgtgtgcctggccggagcgttttgaaacaccgacg

SEQ ID NO: 54 - DNA, 52 bp, synthetic construct
  source 1..52: mol_type = other DNA; note = Probe sequence
cgtcggtcgtccggggccgctcggcggcgctgcgattggccgcgcaccgacg

SEQ ID NO: 55 - DNA, 50 bp, synthetic construct
  source 1..50: mol_type = other DNA; note = Probe sequence
cgtcggtcggggtaacctctatgcaaatgaggccgcgccgcccaccgacg

SEQ ID NO: 56 - DNA, 51 bp, synthetic construct
  source 1..51: mol_type = other DNA; note = Probe sequence
cgtcggtcggcgggctcggcccggtccctccgctggggggttacaccgacg

SEQ ID NO: 57 - DNA, 51 bp, synthetic construct
  source 1..51: mol_type = other DNA; note = Probe sequence
cgtcggtcgagccggccggcagcgagatacccagaggcccgttcaccgacg

SEQ ID NO: 58 - DNA, 51 bp, synthetic construct
  source 1..51: mol_type = other DNA; note = Probe sequence
cgtcggtcgcaccgcgttgccatagcaacggcctggccggctgcaccgacg

SEQ ID NO: 59 - DNA, 52 bp, synthetic construct
  source 1..52: mol_type = other DNA; note = Probe sequence
cgtcggtcggaggtgccggctgcacaacggcgcccacgtgaccccaccgacg

SEQ ID NO: 60 - DNA, 51 bp, synthetic construct
  source 1..51: mol_type = other DNA; note = Probe sequence
cgtcggtcggtgcagccccaggcgcgcccaagggcagctcgcccaccgacg

SEQ ID NO: 61 - DNA, 52 bp, synthetic construct
  source 1..52: mol_type = other DNA; note = Probe sequence
cgtcggtcggagaaggacctaaaaccccgtctggggcacagaggcaccgacg

SEQ ID NO: 62 - DNA, 52 bp, synthetic construct
  source 1..52: mol_type = other DNA; note = Probe sequence
cgtcggtcgacatctggggaaaccgaggcgcagagcgggacggccaccgacg

SEQ ID NO: 63 - DNA, 52 bp, synthetic construct
  source 1..52: mol_type = other DNA; note = Probe sequence
cgtcggtcgtgggcctggcgggaagtcgcgcaaggaggccggcacaccgacg

SEQ ID NO: 64 - DNA, 52 bp, synthetic construct
  source 1..52: mol_type = other DNA; note = Probe sequence
cgtcggtcggggcgcacccggcccaccctgtcccttccaggccgcaccgacg

SEQ ID NO: 65 - DNA, 52 bp, synthetic construct
  source 1..52: mol_type = other DNA; note = Probe sequence
cgtcggtcggctgcagcacaggctgcagggggcgggcagcgccgcaccgacg

SEQ ID NO: 66 - DNA, 51 bp, synthetic construct
  source 1..51: mol_type = other DNA; note = Probe sequence
cgtcggtcgtctagcggggcaggcgagcggagcagcagcgttccaccgacg

SEQ ID NO: 67 - DNA, 52 bp, synthetic construct
  source 1..52: mol_type = other DNA; note = Probe sequence
cgtcggtcgagccccggccgcggcccctgagaggcgcgcactcgcaccgacg

SEQ ID NO: 68 - DNA, 52 bp, synthetic construct
  source 1..52: mol_type = other DNA; note = Probe sequence
cgtcggtcggcctccctgtgccagccggctgtcgacccaggttacaccgacg

SEQ ID NO: 69 - DNA, 52 bp, synthetic construct
  source 1..52: mol_type = other DNA; note = Probe sequence
cgtcggtcgaagcccgaggtcggggcgttaccccaagggccctccaccgacg

SEQ ID NO: 70 - DNA, 52 bp, synthetic construct
  source 1..52: mol_type = other DNA; note = Probe sequence
cgtcggtcggcttcccctccgagggcagagaggcgtccgcgccccaccgacg

SEQ ID NO: 71 - DNA, 52 bp, synthetic construct
  source 1..52: mol_type = other DNA; note = Probe sequence
cgtcggtcgggggctgcggggtccgtggaacctttccgggaggccaccgacg

SEQ ID NO: 72 - DNA, 52 bp, synthetic construct
  source 1..52: mol_type = other DNA; note = Probe sequence
cgtcggtcggccgcgggctgctgggcgcggaggctggagccgcgcaccgacg

SEQ ID NO: 73 - DNA, 52 bp, synthetic construct
  source 1..52: mol_type = other DNA; note = Probe sequence
cgtcggtcgaggttcggctgctgaagcggccactgcctcccagacaccgacg

SEQ ID NO: 74 - DNA, 52 bp, synthetic construct
  source 1..52: mol_type = other DNA; note = Probe sequence
cgtcggtcggatcgatggagagaaggcgggcaagacgccgggaacaccgacg

SEQ ID NO: 75 - DNA, 52 bp, synthetic construct
  source 1..52: mol_type = other DNA; note = Probe sequence
cgtcggtcggcattcctcctcaaccgagtgccacaaccgccctccaccgacg

SEQ ID NO: 76 - DNA, 51 bp, synthetic construct
  source 1..51: mol_type = other DNA; note = Probe sequence
cgtcggtcggaagtgccccggggcttcgagcatcacctcgcggcaccgacg

SEQ ID NO: 77 - DNA, 52 bp, synthetic construct
  source 1..52: mol_type = other DNA; note = Probe sequence
cgtcggtcgagctgagaccggcggccgacggccagccctcagggcaccgacg

SEQ ID NO: 78 - DNA, 51 bp, synthetic construct
  source 1..51: mol_type = other DNA; note = Probe sequence
cgtcggtcgggtcacaagtcagcgcccaagcaagtcaagcgaccaccgacg

SEQ ID NO: 79 - DNA, 51 bp, synthetic construct
  source 1..51: mol_type = other DNA; note = Probe sequence
cgtcggtcggctcgtcttcgcccgaactgatgcgctgcaaacgcaccgacg

SEQ ID NO: 80 - DNA, 52 bp, synthetic construct
  source 1..52: mol_type = other DNA; note = Probe sequence
cgtcggtcgggctcaacttcagcggctttggctacagcctgccgcaccgacg

SEQ ID NO: 81 - DNA, 51 bp, synthetic construct
  source 1..51: mol_type = other DNA; note = Probe sequence
cgtcggtcggagcgcaaccgcgtcaagttggtcaacctgggctcaccgacg

SEQ ID NO: 82 - DNA, 51 bp, synthetic construct
  source 1..51: mol_type = other DNA; note = Probe sequence
cgtcggtcgcacccttcgggagcacgtccccaacggcgcggcccaccgacg

SEQ ID NO: 83 - DNA, 51 bp, synthetic construct
  source 1..51: mol_type = other DNA; note = Probe sequence
cgtcggtcgaagaagatgagtaaggtggagacactgcgctcggcaccgacg

SEQ ID NO: 84 - DNA, 50 bp, synthetic construct
  source 1..50: mol_type = other DNA; note = Probe sequence
cgtcggtcgtggccctggttgggtccgcccgcagcgagggcgcaccgacg

SEQ ID NO: 85 - DNA, 52 bp, synthetic construct
  source 1..52: mol_type = other DNA; note = Probe sequence
cgtcggtcgagacctgcgaagaagttcggaaacttttccagtggcaccgacg

SEQ ID NO: 86 - DNA, 52 bp, synthetic construct
  source 1..52: mol_type = other DNA; note = Probe sequence
cgtcggtcggctgctgggagctgtcagggggctgccggattcgccaccgacg

SEQ ID NO: 87 - DNA, 52 bp, synthetic construct
  source 1..52: mol_type = other DNA; note = Probe sequence
cgtcggtcggccgaggctgggagcgcggtgatggccggtccccgcaccgacg

SEQ ID NO: 88 - DNA, 52 bp, synthetic construct
  source 1..52: mol_type = other DNA; note = Probe sequence
cgtcggtcgagcagagggcagcggcggcgggaccggggactctgcaccgacg

SEQ ID NO: 89 - DNA, 51 bp, synthetic construct
  source 1..51: mol_type = other DNA; note = Probe sequence
cgtcggtcgcaatgggtaaagccaggaggaagcccgtgcctggcaccgacg

SEQ ID NO: 90 - DNA, 52 bp, synthetic construct
  source 1..52: mol_type = other DNA; note = Probe sequence
cgtcggtcgaggcgggcaggaggggaggagtagggaggcgagagcaccgacg

SEQ ID NO: 91 - DNA, 52 bp, synthetic construct
  source 1..52: mol_type = other DNA; note = Probe sequence
cgtcggtcggcgggcgggaggcgccacggcctctcagacgctggcaccgacg

SEQ ID NO: 92 - DNA, 51 bp, synthetic construct
  source 1..51: mol_type = other DNA; note = Probe sequence
cgtcggtcgccgcagccgagaagccagagagaaagttcccgggcaccgacg

SEQ ID NO: 93 - DNA, 51 bp, synthetic construct
  source 1..51: mol_type = other DNA; note = Probe sequence
cgtcggtcggcagtaagcgagtaagcgagccctggagaccgggcaccgacg

SEQ ID NO: 94 - DNA, 51 bp, synthetic construct
  source 1..51: mol_type = other DNA; note = Probe sequence
cgtcggtcgctgggtgtgcggtcggctcagtgccacgcggtgacaccgacg

SEQ ID NO: 95 - DNA, 51 bp, synthetic construct
  source 1..51: mol_type = other DNA; note = Probe sequence
cgtcggtcgtaggcatggttatcaacccacgccaaggcggttgcaccgacg

SEQ ID NO: 96 - DNA, 52 bp, synthetic construct
  source 1..52: mol_type = other DNA; note = Probe sequence
cgtcggtcggctgcctcgccccggagcccggaggaggggagccgcaccgacg

SEQ ID NO: 97 - DNA, 51 bp, synthetic construct
  source 1..51: mol_type = other DNA; note = Probe sequence
cgtcggtcgacccggggaagaagcggaggacgccgatctggcccaccgacg

SEQ ID NO: 98 - DNA, 51 bp, synthetic construct
  source 1..51: mol_type = other DNA; note = Probe sequence
cgtcggtcgtgcgttgcgcgctccaaccctctgcttggccgcccaccgacg

SEQ ID NO: 99 - DNA, 52 bp, synthetic construct
  source 1..52: mol_type = other DNA; note = Probe sequence
cgtcggtcgacaaatccccgaggcggggagactttcagggcatccaccgacg

SEQ ID NO: 100 - DNA, 52 bp, synthetic construct
  source 1..52: mol_type = other DNA; note = Probe sequence
cgtcggtcggatgctgaagcctcgcggtccccattcccaagccccaccgacg

SEQ ID NO: 101 - DNA, 51 bp, synthetic construct
  source 1..51: mol_type = other DNA; note = Probe sequence
cgtcggtcgccgtgcgccgcctgcgcgtggcgcagttaatttgcaccgacg

SEQ ID NO: 102 - DNA, 51 bp, synthetic construct
  source 1..51: mol_type = other DNA; note = Probe sequence
cgtcggtcggtcttgaggtggggaggggagaaatgggaagaggcaccgacg

SEQ ID NO: 103 - DNA, 51 bp, synthetic construct
  source 1..51: mol_type = other DNA; note = Probe sequence
cgtcggtcgagtagcggttttagcccgctctgcggctgcgaggcaccgacg

SEQ ID NO: 104 - DNA, 52 bp, synthetic construct
  source 1..52: mol_type = other DNA; note = Probe sequence
cgtcggtcgagatccgagattaacctctcccgcgataggtgaagcaccgacg

SEQ ID NO: 105 - DNA, 51 bp, synthetic construct
  source 1..51: mol_type = other DNA; note = Probe sequence
cgtcggtcgttggggcgacggggccaggcgcgggggacggctgcaccgacg

SEQ ID NO: 106 - DNA, 52 bp, synthetic construct
  source 1..52: mol_type = other DNA; note = Probe sequence
cgtcggtcgggctgggagggcgcgcggaggagacaccgctgaggcaccgacg

SEQ ID NO: 107 - DNA, 52 bp, synthetic construct
  source 1..52: mol_type = other DNA; note = Probe sequence
cgtcggtcgacgccgctgagggcgccacgcggggggcgcggctgcaccgacg

SEQ ID NO: 108 - DNA, 52 bp, synthetic construct
  source 1..52: mol_type = other DNA; note = Probe sequence
cgtcggtcgagtgcgcacttgaggcgcgggacgcaccggctgtgcaccgacg

SEQ ID NO: 109 - DNA, 52 bp, synthetic construct
  source 1..52: mol_type = other DNA; note = Probe sequence
cgtcggtcgtcccaggggctgagactcgcgccccgccccgcagccaccgacg

SEQ ID NO: 110 - DNA, 52 bp, synthetic construct
  source 1..52: mol_type = other DNA; note = Probe sequence
cgtcggtcgtcggctcgccgggccgggcccctctccggaacctccaccgacg

SEQ ID NO: 111 - DNA, 52 bp, synthetic construct
  source 1..52: mol_type = other DNA; note = Probe sequence
cgtcggtcggcggctggaggacgcgctgctgcggatgcgcgaggcaccgacg

SEQ ID NO: 112 - DNA, 52 bp, synthetic construct
  source 1..52: mol_type = other DNA; note = Probe sequence
cgtcggtcgtacgggatacaggccgaggagcggcaggtccgtgccaccgacg

SEQ ID NO: 113 - DNA, 52 bp, synthetic construct
  source 1..52: mol_type = other DNA; note = Probe sequence
cgtcggtcgggggatggcgcgctgaccccatacccgctgccgtccaccgacg

SEQ ID NO: 114 - DNA, 51 bp, synthetic construct
  source 1..51: mol_type = other DNA; note = Probe sequence
cgtcggtcgcggctgcggggccgccgccgagcgagggcgaggacaccgacg

SEQ ID NO: 115 - DNA, 52 bp, synthetic construct
  source 1..52: mol_type = other DNA; note = Probe sequence
cgtcggtcggcaccgtgcgcttcgcccgcaaaggcgccctccggcaccgacg

SEQ ID NO: 116 - DNA, 52 bp, synthetic construct
  source 1..52: mol_type = other DNA; note = Probe sequence
cgtcggtcggaagaacgtgcatgaggtcaagaaccacaaattcacaccgacg

SEQ ID NO: 117 - DNA, 51 bp, synthetic construct
  source 1..51: mol_type = other DNA; note = Probe sequence
cgtcggtcggatggccgcgccgccccgggggagccggagccgacaccgacg

SEQ ID NO: 118 - DNA, 52 bp, synthetic construct
  source 1..52: mol_type = other DNA; note = Probe sequence
cgtcggtcgtggccgccgcccgcgcgcactcaccaagcccgctgcaccgacg

SEQ ID NO: 119 - DNA, 51 bp, synthetic construct
  source 1..51: mol_type = other DNA; note = Probe sequence
cgtcggtcgtcctcctcgcacgagtaccagatgccggtgtggacaccgacg

SEQ ID NO: 120 - DNA, 52 bp, synthetic construct
  source 1..52: mol_type = other DNA; note = Probe sequence
cgtcggtcgtccctgggccgggactggagcgcaaacggttgggacaccgacg

SEQ ID NO: 121 - DNA, 51 bp, synthetic construct
  source 1..51: mol_type = other DNA; note = Probe sequence
cgtcggtcgtgtcggtgtctgcccgcccgtctgtgcgtctgtccaccgacg

SEQ ID NO: 122 - DNA, 52 bp, synthetic construct
  source 1..52: mol_type = other DNA; note = Probe sequence
cgtcggtcgtgtcggtgtgagcgtctgaggcgatggggaagacacaccgacg

SEQ ID NO: 123 - DNA, 51 bp, synthetic construct
  source 1..51: mol_type = other DNA; note = Probe sequence
cgtcggtcggggcgcttctagtcggacaaaatgcagccgagaacaccgacg

SEQ ID NO: 124 - DNA, 51 bp, synthetic construct
  source 1..51: mol_type = other DNA; note = Probe sequence
cgtcggtcgcgctcgttctgtgcgttctcctgtcccaggtaggcaccgacg

SEQ ID NO: 125 - DNA, 52 bp, synthetic construct
  source 1..52: mol_type = other DNA; note = Probe sequence
cgtcggtcgagaggggctgccgggcgcgctctgcgccccgtttccaccgacg

SEQ ID NO: 126 - DNA, 51 bp, synthetic construct
  source 1..51: mol_type = other DNA; note = Probe sequence
cgtcggtcgtgggagcagggtgtccgaagcgcgggtaccgatccaccgacg

SEQ ID NO: 127 - DNA, 52 bp, synthetic construct
  source 1..52: mol_type = other DNA; note = Probe sequence
cgtcggtcgggcagcgcggggcacgcggcgcgcgggcgagtctgcaccgacg

SEQ ID NO: 128 - DNA, 51 bp, synthetic construct
  source 1..51: mol_type = other DNA; note = Probe sequence
cgtcggtcgtgcgcgcgcggacgccttggttcccggagcccagcaccgacg

SEQ ID NO: 129 - DNA, 51 bp, synthetic construct
  source 1..51: mol_type = other DNA; note = Probe sequence
cgtcggtcgccaccttctcagtccgggacgcgagacgggaacgcaccgacg

SEQ ID NO: 130 - DNA, 51 bp, synthetic construct
  source 1..51: mol_type = other DNA; note = Probe sequence
cgtcggtcggccctggcgccccaacgctgcaccaccgtgggtccaccgacg

SEQ ID NO: 131 - DNA, 52 bp, synthetic construct
  source 1..52: mol_type = other DNA; note = Probe sequence
cgtcggtcggagccgtgctcgcagtcgctgagatcctcggtgcgcaccgacg

SEQ ID NO: 132 - DNA, 52 bp, synthetic construct
  source 1..52: mol_type = other DNA; note = Probe sequence
cgtcggtcggcgtctctcgccgtcccctgggcgcgggccaggcgcaccgacg

SEQ ID NO: 133 - DNA, 51 bp, synthetic construct
  source 1..51: mol_type = other DNA; note = Probe sequence
cgtcggtcggaggaggggggcgctccggtcgtgtgcccaggaccaccgacg

SEQ ID NO: 134 - DNA, 51 bp, synthetic construct
  source 1..51: mol_type = other DNA; note = Probe sequence
cgtcggtcgccccagcggccactcgggccccagccccccaggccaccgacg

SEQ ID NO: 135 - DNA, 52 bp, synthetic construct
  source 1..52: mol_type = other DNA; note = Probe sequence
cgtcggtcgtggagatttagagcccgggaatgaggcgccgtgtccaccgacg

SEQ ID NO: 136 - DNA, 52 bp, synthetic construct
  source 1..52: mol_type = other DNA; note = Probe sequence
cgtcggtcgtaggaatctcgcgcccggggagcgctgagggaccgcaccgacg

SEQ ID NO: 137 - DNA, 52 bp, synthetic construct
  source 1..52: mol_type = other DNA; note = Probe sequence
cgtcggtcggagccgggtggggagcgggcctcggggcgcccggccaccgacg

SEQ ID NO: 138 - DNA, 52 bp, synthetic construct
  source 1..52: mol_type = other DNA; note = Probe sequence
cgtcggtcggcagggccggaaggaggcccctgccccgtccaaggcaccgacg

SEQ ID NO: 139 - DNA, 52 bp, synthetic construct
  source 1..52: mol_type = other DNA; note = Probe sequence
cgtcggtcggcaccagctgccccgccgcccgcccggacccagcccaccgacg

SEQ ID NO: 140 - DNA, 52 bp, synthetic construct
  source 1..52: mol_type = other DNA; note = Probe sequence
cgtcggtcggcctcattgctgacgagaccccgccctgctactcccaccgacg

SEQ ID NO: 141 - DNA, 52 bp, synthetic construct
  source 1..52: mol_type = other DNA; note = Probe sequence
cgtcggtcgggccggagaaggcgccgctggggccgcccggaggacaccgacg

SEQ ID NO: 142 - DNA, 50 bp, synthetic construct
  source 1..50: mol_type = other DNA; note = Probe sequence
cgtcggtcgcctctgcacgggcccgtggagacgcttcctgcgcaccgacg

SEQ ID NO: 143 - DNA, 52 bp, synthetic construct
  source 1..52: mol_type = other DNA; note = Probe sequence
cgtcggtcgaaccttctggaatccaccgcccccctttccgcccgcaccgacg

SEQ ID NO: 144 - DNA, 51 bp, synthetic construct
  source 1..51: mol_type = other DNA; note = Probe sequence
cgtcggtcgcgcgcccgcccccaggagggcctccgcgagccggcaccgacg

SEQ ID NO: 145 - DNA, 52 bp, synthetic construct
  source 1..52: mol_type = other DNA; note = Probe sequence
cgtcggtcggcacaccccgaggcggtcccggctgcacaacttggcaccgacg

SEQ ID NO: 146 - DNA, 51 bp, synthetic construct
  source 1..51: mol_type = other DNA; note = Probe sequence
cgtcggtcggagttgctccgtttcctcattttgggggcgaagacaccgacg

SEQ ID NO: 147 - DNA, 52 bp, synthetic construct
  source 1..52: mol_type = other DNA; note = Probe sequence
cgtcggtcggccggcggcggccagtagcggcgccgtgtgcagggcaccgacg

SEQ ID NO: 148 - DNA, 52 bp, synthetic construct
  source 1..52: mol_type = other DNA; note = Probe sequence
cgtcggtcgagcgccgcctgcgccgcgttcagcacgaagagctccaccgacg

SEQ ID NO: 149 - DNA, 52 bp, synthetic construct
  source 1..52: mol_type = other DNA; note = Probe sequence
cgtcggtcgtccagctcaggcgcagcagcgccacctggtcggcccaccgacg

SEQ ID NO: 150 - DNA, 52 bp, synthetic construct
  source 1..52: mol_type = other DNA; note = Probe sequence
cgtcggtcgggcgcccgcattggtgctgacataatttcctgacccaccgacg

SEQ ID NO: 151 - DNA, 53 bp, synthetic construct
  source 1..53: mol_type = other DNA; note = Probe sequence
cgtcggtcgtgacccgtattgtctcgcgattaaaggtaaaaaacgcaccgacg

SEQ ID NO: 152 - DNA, 52 bp, synthetic construct
  source 1..52: mol_type = other DNA; note = Probe sequence
cgtcggtcggctttttcatcccactggggtaaaacgcccttttacaccgacg

SEQ ID NO: 153 - DNA, 52 bp, synthetic construct
  source 1..52: mol_type = other DNA; note = Probe sequence
cgtcggtcgagtggggccgcggggcctgctgggaggtgttgtcccaccgacg

SEQ ID NO: 154 - DNA, 52 bp, synthetic construct
  source 1..52: mol_type = other DNA; note = Probe sequence
cgtcggtcgggaaacgtcgctggcgcggagggatggttcggcgccaccgacg

SEQ ID NO: 155 - DNA, 51 bp, synthetic construct
  source 1..51: mol_type = other DNA; note = Probe sequence
cgtcggtcgtaggcgtctgtcacagacctatctgcgggtcgcccaccgacg

SEQ ID NO: 156 - DNA, 50 bp, synthetic construct
  source 1..50: mol_type = other DNA; note = Probe sequence
cgtcggtcgccagcgccatagcccttaggactatcggtcacacaccgacg

SEQ ID NO: 157 - DNA, 50 bp, synthetic construct
  source 1..50: mol_type = other DNA; note = Probe sequence
cgtcggtcctcgcgctcctgctccggctcctccatcttggcccaccgacg

SEQ ID NO: 158 - DNA, 50 bp, synthetic construct
  source 1..50: mol_type = other DNA; note = Probe sequence
cgtcggtcggagcagagcgaggtgtgtgcctccttaccgcctcaccgacg

SEQ ID NO: 159 - DNA, 51 bp, synthetic construct
  source 1..51: mol_type = other DNA; note = Probe sequence
cgtcggtcgtgcactggacgtccttccccagcagccagttgagcaccgacg

SEQ ID NO: 160 - DNA, 51 bp, synthetic construct
  source 1..51: mol_type = other DNA; note = Probe sequence
cgtcggtcagacggaggctggtggtgcagcaggcaggcaagaccaccgacg

SEQ ID NO: 161 - DNA, 51 bp, synthetic construct
  source 1..51: mol_type = other DNA; note = Probe sequence
cgtcggtcgatgccggggactacagctgcgaggccaggggccacaccgacg

SEQ ID NO: 162 - DNA, 51 bp, synthetic construct
  source 1..51: mol_type = other DNA; note = Probe sequence
cgtcggtcgcacagcgttgtgcatccaggtctagcgtgtcttccaccgacg

SEQ ID NO: 163 - DNA, 55 bp, synthetic construct
  source 1..55: mol_type = other DNA; note = Probe sequence
cgtcggtcctgtcttctgtggatgaggtatatgaatttatcccaaagcaccgacg

SEQ ID NO: 164 - DNA, 51 bp, synthetic construct
  source 1..51: mol_type = other DNA; note = Probe sequence
cgtcggtccgagacctcccagagcccgtggttccctggagccacaccgacg

SEQ ID NO: 165 - DNA, 51 bp, synthetic construct
  source 1..51: mol_type = other DNA; note = Probe sequence
cgtcggtctacgaagggttcctgctctgtgggcagctcacgaacaccgacg

SEQ ID NO: 166 - DNA, 56 bp, synthetic construct
  source 1..56: mol_type = other DNA; note = Probe sequence
cgtcggtccaataatgcacatggagaaagttcacctacaataaagaggcaccgacg

SEQ ID NO: 167 - DNA, 55 bp, synthetic construct
  source 1..55: mol_type = other DNA; note = Probe sequence
cgtcggtctgtattggtaacattttatatcgaattcctgttctatgtcaccgacg

SEQ ID NO: 168 - DNA, 51 bp, synthetic construct
  source 1..51: mol_type = other DNA; note = Probe sequence
cgtcggtcagatgtcccctccctgtccgtccccgcacctggagcaccgacg

SEQ ID NO: 169 - DNA, 51 bp, synthetic construct
  source 1..51: mol_type = other DNA; note = Probe sequence
cgtcggtctggtggtgcatgcccgaacccagcacttccttgaacaccgacg

SEQ ID NO: 170 - DNA, 50 bp, synthetic construct
  source 1..50: mol_type = other DNA; note = Probe sequence
cgtcggtccaactggccaacctagagcccccctggtaaaagccaccgacg

SEQ ID NO: 171 - DNA, 55 bp, synthetic construct
  source 1..55: mol_type = other DNA; note = Probe sequence
cgtcggtctcttggtggaatagatgttaattagtttttttattactccaccgacg

SEQ ID NO: 172 - DNA, 51 bp, synthetic construct
  source 1..51: mol_type = other DNA; note = Probe sequence
cgtcggtcggaaacaattctgtgttcaccctcaccctgcaggccaccgacg

SEQ ID NO: 173 - DNA, 51 bp, synthetic construct
  source 1..51: mol_type = other DNA; note = Probe sequence
cgtcggtcggcctctcagccatcaagacaccgtatcctacctccaccgacg

SEQ ID NO: 174 - DNA, 51 bp, synthetic construct
  source 1..51: mol_type = other DNA; note = Probe sequence
cgtcggtcacgtgctgagcgcacgcacgtggcgcctgctcacccaccgacg

SEQ ID NO: 175 - DNA, 51 bp, synthetic construct
  source 1..51: mol_type = other DNA; note = Probe sequence
cgtcggtcgatgctgctccagcgcccgcgcgagttgcggatcgcaccgacg

SEQ ID NO: 176 - DNA, 56 bp, synthetic construct
  source 1..56: mol_type = other DNA; note = Probe sequence
cgtcggtcgtagttgacaaatacatttagtgatgtcttacttttttggcaccgacg

SEQ ID NO: 177 - DNA, 51 bp, synthetic construct
  source 1..51: mol_type = other DNA; note = Probe sequence
cgtcggtcatctcctaccagtgtatccttcacgacagacgcaccaccgacg

SEQ ID NO: 178 - DNA, 51 bp, synthetic construct
  source 1..51: mol_type = other DNA; note = Probe sequence
cgtcggtccgagcgatgatgacaccaaatccatgtgtccaccccaccgacg

SEQ ID NO: 179 - DNA, 50 bp, synthetic construct
  source 1..50: mol_type = other DNA; note = Probe sequence
cgtcggtcgggacccaggagggcacagccaaggaatgagccccaccgacg

SEQ ID NO: 180 - DNA, 51 bp, synthetic construct
  source 1..51: mol_type = other DNA; note = Probe sequence
cgtcggtcctcctggtcagcagcctcttagagaacctgctggacaccgacg

SEQ ID NO: 181 - DNA, 52 bp, synthetic construct
  source 1..52: mol_type = other DNA; note = Probe sequence
cgtcggtctatagaaccatcatcatgcaagatgagagcaaggagcaccgacg

SEQ ID NO: 182 - DNA, 56 bp, synthetic construct
  source 1..56: mol_type = other DNA; note = Probe sequence
cgtcggtcgaacagtaaacagtggttctgactggtgaaatgatagttacaccgacg

SEQ ID NO: 183 - DNA, 55 bp, synthetic construct
  source 1..55: mol_type = other DNA; note = Probe sequence
cgtcggtcgttgaaaggaccagcactttatttattgctttagccattcaccgacg

SEQ ID NO: 184 - DNA, 51 bp, synthetic construct
  source 1..51: mol_type = other DNA; note = Probe sequence
cgtcggtcagcctgcacgggagtcagaggcactcagcaatgcccaccgacg

SEQ ID NO: 185 - DNA, 50 bp, synthetic construct
  source 1..50: mol_type = other DNA; note = Probe sequence
cgtcggtctggctctgttacgaacggctgaaatcaaaacccccaccgacg

SEQ ID NO: 186 - DNA, 51 bp, synthetic construct
  source 1..51: mol_type = other DNA; note = Probe sequence
cgtcggtctcaccgtgttctccagaccatgcatgttcctccgccaccgacg

SEQ ID NO: 187 - DNA, 51 bp, synthetic construct
  source 1..51: mol_type = other DNA; note = Probe sequence
cgtcggtcaccgccccttcagggatggggctgtaggagtcaagcaccgacg

SEQ ID NO: 188 - DNA, 51 bp, synthetic construct
  source 1..51: mol_type = other DNA; note = Probe sequence
cgtcggtctctcggtgtctccccaggtgcaagtgcaacctgcacaccgacg

SEQ ID NO: 189 - DNA, 51 bp, synthetic construct
  source 1..51: mol_type = other DNA; note = Probe sequence
cgtcggtcgccaacctgtgctccatgcgcgagggcagcctgcacaccgacg

SEQ ID NO: 190 - DNA, 51 bp, synthetic construct
  source 1..51: mol_type = other DNA; note = Probe sequence
cgtcggtcaagcccactcttctactccccgaacgtgccttccccaccgacg

SEQ ID NO: 191 - DNA, 51 bp, synthetic construct
  source 1..51: mol_type = other DNA; note = Probe sequence
cgtcggtcctctgacggcgacagtagctccgtggacagcgatgcaccgacg

SEQ ID NO: 192 - DNA, 51 bp, synthetic construct
  source 1..51: mol_type = other DNA; note = Probe sequence
cgtcggtcctggaggagcacggaaaagacctggaaatcatgcacaccgacg

SEQ ID NO: 193 - DNA, 51 bp, synthetic construct
  source 1..51: mol_type = other DNA; note = Probe sequence
cgtcggtcatcctcaccagggtgaatgacagagttgccaggcacaccgacg

SEQ ID NO: 194 - DNA, 51 bp, synthetic construct
  source 1..51: mol_type = other DNA; note = Probe sequence
cgtcggtcgcataggagtaggccagccagcggaacacgtggtccaccgacg

SEQ ID NO: 195 - DNA, 51 bp, synthetic construct
  source 1..51: mol_type = other DNA; note = Probe sequence
cgtcggtctcgggggtgggggtgtgttcctgcgtcttccagggcaccgacg

SEQ ID NO: 196 - DNA, 51 bp, synthetic construct
  source 1..51: mol_type = other DNA; note = Probe sequence
cgtcggtccgggaatgccgagtaagtgttaattttatggtccccaccgacg

SEQ ID NO: 197 - DNA, 56 bp, synthetic construct
  source 1..56: mol_type = other DNA; note = Probe sequence
cgtcggtcatcacttctggaaaatgaatagatagatgtgtgggctttacaccgacg

SEQ ID NO: 198 - DNA, 54 bp, synthetic construct
  source 1..54: mol_type = other DNA; note = Probe sequence
cgtcggtcgtgcctcaatgatcttttttccccaccttcatttttctcaccgacg

SEQ ID NO: 199 - DNA, 50 bp, synthetic construct
  source 1..50: mol_type = other DNA; note = Probe sequence
cgtcggtccttcagcggcatctgctagctcgtctacccctgtcaccgacg

SEQ ID NO: 200 - DNA, 54 bp, synthetic construct
  source 1..54: mol_type = other DNA; note = Probe sequence
cgtcggtccatgttttagggaactctgccctataaacactcatagacaccgacg

SEQ ID NO: 201 - DNA, 51 bp, synthetic construct
  source 1..51: mol_type = other DNA; note = Probe sequence
cgtcggtcggtttctctctatgttgcagtccctctgtcgtgaacaccgacg

SEQ ID NO: 202 - DNA, 50 bp, synthetic construct
  source 1..50: mol_type = other DNA; note = Probe sequence
cgtcggtccggcattcctgtggtagtggcctgagaacacgaccaccgacg

SEQ ID NO: 203 - DNA, 51 bp, synthetic construct
  source 1..51: mol_type = other DNA; note = Probe sequence
cgtcggtctgacacctgcagagaagggaaaaagtcattaggggcaccgacg

SEQ ID NO: 204 - DNA, 51 bp, synthetic construct
  source 1..51: mol_type = other DNA; note = Probe sequence
cgtcggtcacatgtccctgcgtcacaggcacctgcagagcccccaccgacg

SEQ ID NO: 205 - DNA, 51 bp, synthetic construct
  source 1..51: mol_type = other DNA; note = Probe sequence
cgtcggtctgtgtaaggcgttccggcacgtcaaggtggacacacaccgacg

SEQ ID NO: 206 - DNA, 51 bp, synthetic construct
  source 1..51: mol_type = other DNA; note = Probe sequence
cgtcggtctgaagatacaaacaaccacagcagcctgcacttaccaccgacg

SEQ ID NO: 207 - DNA, 51 bp, synthetic construct
  source 1..51: mol_type = other DNA; note = Probe sequence
cgtcggtcgtgtggtcatcttcttcttccccttctagcacgaccaccgacg

SEQ ID NO: 208 - DNA, 51 bp, synthetic construct
  source 1..51: mol_type = other DNA; note = Probe sequence
cgtcggtcacgttgcatcgaccctctccactccgcggaagtagcaccgacg

SEQ ID NO: 209 - DNA, 50 bp, synthetic construct
  source 1..50: mol_type = other DNA; note = Probe sequence
cgtcggtccgacaccgtctgatgtgttgcgcaggtggtggcacaccgacg

SEQ ID NO: 210 - DNA, 51 bp, synthetic construct
  source 1..51: mol_type = other DNA; note = Probe sequence
cgtcggtccattgggatggagggtggggaaggagtcaccctggcaccgacg

SEQ ID NO: 211 - DNA, 50 bp, synthetic construct
  source 1..50: mol_type = other DNA; note = Probe sequence
cgtcggtccctcctccgcctgacttacttgatcctaaagtcacaccgacg

SEQ ID NO: 212 - DNA, 50 bp, synthetic construct
  source 1..50: mol_type = other DNA; note = Probe sequence
cgtcggtcctcccagggctccttggcctcctccgcggtgacccaccgacg

SEQ ID NO: 213 - DNA, 51 bp, synthetic construct
  source 1..51: mol_type = other DNA; note = Probe sequence
cgtcggtcgggacacagggccgcatgagcctgggcggggtcagcaccgacg

SEQ ID NO: 214 - DNA, 51 bp, synthetic construct
  source 1..51: mol_type = other DNA; note = Probe sequence
cgtcggtccgccctccgaggagggcccgggcggggtgggcgcccaccgacg

SEQ ID NO: 215 - DNA, 50 bp, synthetic construct
  source 1..50: mol_type = other DNA; note = Probe sequence
cgtcggtccgtcctcaggctccaggctgggaggagagagcgtcaccgacg

SEQ ID NO: 216 - DNA, 51 bp, synthetic construct
  source 1..51: mol_type = other DNA; note = Probe sequence
cgtcggtcgctgggagtggagctgggggtcagaagagcaagcacaccgacg

SEQ ID NO: 217 - DNA, 54 bp, synthetic construct
  source 1..54: mol_type = other DNA; note = Probe sequence
cgtcggtcaacgaaattgatcaaacttagactgcttcacctgtctccaccgacg

SEQ ID NO: 218 - DNA, 51 bp, synthetic construct
  source 1..51: mol_type = other DNA; note = Probe sequence
cgtcggtcgcgtggacaggcagcgccgcagtgacgtctccatgcaccgacg

SEQ ID NO: 219 - DNA, 51 bp, synthetic construct
  source 1..51: mol_type = other DNA; note = Probe sequence
cgtcggtctggagtcctccagcggcttcaggcggttcagcttccaccgacg